European Patent Application EP 4 202 061 A1, published June 28, 2023. Title: BIOMARKER FOR DIAGNOSING AGE-RELATED MACULAR DEGENERATION AND USES THEREOF. Applicant: Genome Opinion Inc. SEOUL NATIONAL UNIVERSITY HOSPITAL. The sequence listing filed with the application follows.

SEQUENCE LISTING (65 sequences)

SEQ ID NO: 1 - DNA, 120 bp, Artificial Sequence
  artificial sequence
ccagcactcaccctgccctctctgccttttctcccccagggtatttggtttcccagtccactatactgacgtctccaacatgagccgcttggcgaggcagagactgctgggccggtcatg

SEQ ID NO: 2 - DNA, 120 bp, Artificial Sequence; identical to SEQ ID NO: 1
  artificial sequence

SEQ ID NO: 3 - DNA, 120 bp, Artificial Sequence
  artificial sequence
ttcagcaaagtgaggaccattactacgaggtcaaactccataaagcagggcaaagaccagcattttcctgtcttcatgaatgagaaagaggacatcttatggtgcactgaaatggaaagg

SEQ ID NO: 4 - DNA, 120 bp, Artificial Sequence
  artificial sequence
ttacagtctctcttctgcctcctaggccgttggcatccactgtgaatgataagctggagctgcaggagtgtctggagcatggcaggatagccaaggtcagctccagcgtctagaacctct

SEQ ID NO: 5 - DNA, 120 bp, Artificial Sequence
  artificial sequence
cgtctcctgttttgtagtccaaccctgtgatgattgatgccaaagaagtgtcagctgcacacagggcccgctacttctggggtaaccttcccggtatgaacaggttggtgaaagctcctg

SEQ ID NO: 6 - DNA, 120 bp, Artificial Sequence; identical to SEQ ID NO: 5
  artificial sequence

SEQ ID NO: 7 - DNA, 120 bp, Artificial Sequence
  artificial sequence
cccttcttctggctctttgagaatgtggtggccatgggcgttagtgacaagagggacatctcgcgatttctcgaggtatagccagcaaccttggtttggccagctcactaatggcttcta

SEQ ID NO: 8 - DNA, 120 bp, Artificial Sequence
  artificial sequence
ctatgcagacagccccagctgatggctttctcttccgacctctcagagggcactggccggctcttctttgagttctaccgcctcctgcatgatgcgcggcccaaggagggagatgatcgc

SEQ ID NO: 9 - DNA, 120 bp, Artificial Sequence; identical to SEQ ID NO: 8
  artificial sequence

SEQ ID NO: 10 - DNA, 120 bp, Artificial Sequence
  artificial sequence
ctttatcctcccagatccaggagtggggcccattcgatctggtgattgggggcagtccctgcaatgacctctccatcgtcaaccctgctcgcaagggcctctacggtaggtaccatcctg

SEQ ID NO: 11 - DNA, 120 bp, Artificial Sequence
  artificial sequence
cacggtgggcatggtgcggcaccaggggaagatcatgtacgtcggggacgtccgcagcgtcacacagaagcatgtatgtccatgctgtggggcgcagcccgtcttcccctccctgcacac

SEQ ID NO: 12 - DNA, 120 bp, Artificial Sequence
  artificial sequence
ccagggagatggctccaagtaacggtgctgtctgctggctggtgcagggctcctggtgctgaaggacttgggcattcaggtggaccgctacattgcctcggaggtgtgtgaggactccat

SEQ ID NO: 13 - DNA, 120 bp, Artificial Sequence; identical to SEQ ID NO: 12
  artificial sequence

SEQ ID NO: 14 - DNA, 120 bp, Artificial Sequence
  artificial sequence
ggcacaagggtacctacgggctgctgcggcggcgagaggactggccctcccggctccagatgttcttcgctaataaccacgaccaggaatttgtgagtgctgggcctggggcgcggtctc

SEQ ID NO: 15 - DNA, 120 bp, Artificial Sequence
  artificial sequence
gtgcagaacaagcccatgattgaatgggccctggggggcttccagccttctggccctaagggcctggagccaccagaaggtaaatgagggcacccagctttctgggacccctgcccgcca

SEQ ID NO: 16 - DNA, 120 bp, Artificial Sequence
  artificial sequence
ttggtggatgacgggccggagccgagcagctgaaggcacccgctgggtcatgtggttcggagacggcaaattctcagtggtaagttgtggggtttggcagtagcctggggtgggggaagg

SEQ ID NO: 17 - DNA, 120 bp, Artificial Sequence; identical to SEQ ID NO: 16
  artificial sequence

SEQ ID NO: 18 - DNA, 120 bp, Artificial Sequence
  artificial sequence
gtgaccactgtgtaatgatttctgctccttggggctccaggacggccggggctttggcattggggagctggtgtgggggaaactgcggggcttctcctggtggccaggccgcattgtgtc

SEQ ID NO: 19 - DNA, 120 bp, Artificial Sequence
  artificial sequence
gactggcgccaggaccctcgcagacattaaagcccgtgctctgcaggtccgaggggcgagaggtcaccactgccatagagaggcggccaccactgccatcggaggggggggtggcccggg

SEQ ID NO: 20 - DNA, 120 bp, Artificial Sequence
  artificial sequence
aagctgcctactacagagggctacagttggactcacagatgggctaggagatgcctcccaactccccgttgctcccactggggaccagccatgccaggccttgcccctactgtcctccca

SEQ ID NO: 21 - DNA, 120 bp, Artificial Sequence
  artificial sequence
aacctcagtagctgagagattagtggagcagcctcagttgcatccggatgttagaactgaatgtgagtctggcaccacttcctgggaaagtgatgatgaggagcaaggacccaccgttcc

SEQ ID NO: 22 - DNA, 120 bp, Artificial Sequence
  artificial sequence
acctgaatcctcaccgactgattgcctgcagaacagagcatttgatgacgaattagggcttggtggctcatgccctcctatgagggaaagtgatactagacaagaaaacttgaaaaccaa

SEQ ID NO: 23 - DNA, 120 bp, Artificial Sequence
  artificial sequence
tgtgagtcctgactttacacaagaaagtagagggtattccaagtgtttgcaaaatggaggaataaaacgcacagttagtgaaccttctctctctgggctccttcagatcaagaaattgaa

SEQ ID NO: 24 - DNA, 120 bp, Artificial Sequence
  artificial sequence
acaagaccaaaaggctaatggagaaagacgtaacttcggggtaagccaagaaagaaatccaggtgaaagcagtcaaccaaatgtctccgatttgagtgataagaaagaatctgtgagttc

SEQ ID NO: 25 - DNA, 120 bp, Artificial Sequence
  artificial sequence
gatcaattccgcacagacctctaactctgagctgcctccaaagccagctgcagtggtgagtgaggcctgtgatgctgatgatgctgataatgccagtaaactagctgcaatgctaaatac

SEQ ID NO: 26 - DNA, 120 bp, Artificial Sequence
  artificial sequence
ttgttcaaacaatacacacctagtttcagagaataaagaacagactacacatcctgaactttttgcaggaaacaagacccaaaacttgcatcacatgcaatattttccaaataatgtgat

SEQ ID NO: 27 - DNA, 120 bp, Artificial Sequence
  artificial sequence
acttgatagccacaccccagctttagagcagcaaacaacttcttcagaaaagacaccaaccaaaagaacagctgcttctgttctcaataattttatagagtcaccttccaaattactaga

SEQ ID NO: 28 - DNA, 120 bp, Artificial Sequence
  artificial sequence
aggagcaggtcctaatgtggcagctattagagaaatcatggaagaaaggtaattaacgcaaaggcacagggcagattaacgtttatccttttgtatatgtcagaatttttccagccttca

SEQ ID NO: 29 - DNA, 120 bp, Artificial Sequence
  artificial sequence
atggtgatccacgcaggtggttcgcagaagcagcagtgaagagaagctactgtgtttggtgcgggagcgagctggccacacctgtgaggctgcagtgattgtgattctcatcctggtgtg

SEQ ID NO: 30 - DNA, 120 bp, Artificial Sequence
  artificial sequence
ggaaggaatcccgctgtctctggctgacaaactctactcggagcttaccgagacgctgaggaaatacggcacgctcaccaatcgccggtgtgccttgaatgaagagtaagtgaagcccag

SEQ ID NO: 31 - DNA, 120 bp, Artificial Sequence; identical to SEQ ID NO: 30
  artificial sequence

SEQ ID NO: 32 - DNA, 120 bp, Artificial Sequence
  artificial sequence
attcactttatacaggaagagaaactggagtctcatttgcaaaacctgtccactcttatggcaccaacatataagaaacttgcacctgatgcatataataatcaggtaagtttaaataat

SEQ ID NO: 33 - DNA, 120 bp, Artificial Sequence
  artificial sequence
ctcaggaggagaaaaaacggagtggtgccattcaggtactgagttcttttcggcgaaaagtcaggatgttagcagagccagtcaagacttgccgacaaaggaaactagaagccaagaaag

SEQ ID NO: 34 - DNA, 120 bp, Artificial Sequence
  artificial sequence
gagaccccagcagcagcagccacatcaccctcagacagagtctgtcaactcttattctgcttctggatccaccaatccatacatgagacggcccaatccagttagtccttatccaaactc

SEQ ID NO: 35 - DNA, 120 bp, Artificial Sequence
  artificial sequence
tctggatcctgacattgggggagtggccgtggctccaactcatgggtcaattctcattgagtgtgcaaagcgtgagctgcatgccacaacccctttaaagaatcccaataggaatcaccc

SEQ ID NO: 36 - DNA, 120 bp, Artificial Sequence
  artificial sequence
ccccaccaggatctccctcgtcttttaccagcataagagcatgaatgagccaaaacatggcttggctctttgggaagccaaaatggctgaaaaagcccgtgagaaagaggaagagtgtga

SEQ ID NO: 37 - DNA, 120 bp, Artificial Sequence
  artificial sequence
atagttgttcctgaaaatgataggcccaacccatggccagatgacagtcacaagacttgtgaatacgttaaaagaaggaaaacgcctgccgtgcccacctaactgtccagatgaggtatc

SEQ ID NO: 38 - DNA, 120 bp, Artificial Sequence
  artificial sequence
ttttttttttccttagtctttctttgaagcagcaagtatgatgagcaagctttctcacaagcatttggttttaaattatggagtatgtgtctgtggagacgagagtaagtaaaactacag

SEQ ID NO: 39 - DNA, 120 bp, Artificial Sequence
  artificial sequence
tgacttataatgtaacagcttgttgacccatttgtttttttcagccctcatgatgtattggctacacttctgaacaacctcaaagttcaagaaaggcagaacagagtttgtaccactgta

SEQ ID NO: 40 - DNA, 120 bp, Artificial Sequence
  artificial sequence
gccagttccgtctgtgtgttcgagtggacaaaatggcgaagatcgccaagactcacgaaggtaagcggtctttccctgcttacgtgttttcttcgttgctagcctaataaaagccttttt

SEQ ID NO: 41 - DNA, 120 bp, Artificial Sequence
  artificial sequence
acatctccaggtagacagatgagccaacagaaccttaccaaacaaacaggtttatccaagaatgccagtagtattccaagaagtgagtctgcctccaaaggactaaatcagatgaataat

SEQ ID NO: 42 - DNA, 120 bp, Artificial Sequence
  artificial sequence
cgctttctgccatgatgattgcatcggcccctccaaactgtgcgtctcctgccttgtcgttcggtaatgagactagaaagagatacactgtaaaggagggggaagggaagggttgaccag

SEQ ID NO: 43 - DNA, 120 bp, Artificial Sequence
  artificial sequence
cacacttagcaggttgcaggccattggagagctggaaagcattggggagcttttctcaaggtatgtaattcgtatgactttgttatcctaaagtgcagcttttctgttaccaatagtgac

SEQ ID NO: 44 - DNA, 120 bp, Artificial Sequence
  artificial sequence
ccactgctgaaaagaacagataaataccgaacatacagcaagaaacactttcggattttcagggtaggtaatgaatacccatgtatctaggagagctggtaatttggtcattgtttttag

SEQ ID NO: 45 - DNA, 120 bp, Artificial Sequence
  artificial sequence
aaaccatcgaagacctcgccacccagctcaacctgaaaaccagcaccgtcatcaactggttccacaactacaggtacgacggctggctcacagggagcgccggtcggcccaggggaaggg

SEQ ID NO: 46 - DNA, 120 bp, Artificial Sequence
  artificial sequence
gaattggctctgctcttccaggtttgttgaatgtacagagtgcggaagaaagatgcatcagatctgtgtccttcaccatgagatcatctggcctgctgggtaagtcttaacgttgttact

SEQ ID NO: 47 - DNA, 120 bp, Artificial Sequence
  artificial sequence
tttattctctagcatctattgctggcaccatctgacgtggcaggctgggggatttttatcaaagatcctgtgcagaaaaatgaattcatctcagaatactgtggagaggtaaggcactga

SEQ ID NO: 48 - DNA, 120 bp, Artificial Sequence
  artificial sequence
ttcaagatcacaaacaacatcgacccagtgggaagaatccaaatgcgcacgaggaggacactgcgggggcacctggccaagatctacgccatgcactggggcacagactccaggtaggcg

SEQ ID NO: 49 - DNA, 120 bp, Artificial Sequence
  artificial sequence
gggccagcaggtgagctccatgccaaggtcccaagtgggcagccccccaattttgtccggtcccctgggacgggtgcatttgtgggcaccccctctcccatgcgtttcactttccctcag

SEQ ID NO: 50 - DNA, 120 bp, Artificial Sequence
  artificial sequence
cctgtgcctgaggagccatgcttgtccccccaacctgaggaatcacacctgtccccccagtctgaggagccatgcctgtccccccggcctgaggaatcgcatctgtcccctgagcttgag

SEQ ID NO: 51 - DNA, 120 bp, Artificial Sequence
  artificial sequence
attaaccttatgtgtgacatgttctaatatagtcacattttcattatttttattataaggcctgctgaaaatgactgaatataaacttgtggtagttggagctggtggcgtaggcaagag

SEQ ID NO: 52 - DNA, 120 bp, Artificial Sequence
  artificial sequence
ttatatctgcattaggttattgatgatgctagtaacaatgaactttatgttactgcagctcacaaatgcttttttacatctgcaagaaattaactagtcatcaaatgcttagtagcacag

SEQ ID NO: 53 - DNA, 120 bp, Artificial Sequence
  artificial sequence
tgtcagtgcttcagtaaagcttatttatttatttttttctagcaggcagatagaagttcctgtcactttctccttttttacggggtaggatgtgatattccttctagtggaaataccagt

SEQ ID NO: 54 - DNA, 120 bp, Artificial Sequence
  artificial sequence
ttctcccagcctatcatcctttcccagcctctgtgggcaagtaccccacacccccttcacagcacagttatgcttcctcaaatgctgctgagcgaacacccagtcacagtggtcacctcc

SEQ ID NO: 55 - DNA, 120 bp, Artificial Sequence
  artificial sequence
gccagattgatagggagcattgttttcacctttcaggctgaagatgaggccttactctcagaagaagatgaccccattgatcgacggccatggacacagcagcaccttgaagctgcagac

SEQ ID NO: 56 - DNA, 120 bp, Artificial Sequence
  artificial sequence
attagaagagtccaattctggccccctgatgaagaagcatagacgaaatggcttaagtcgaagtagtggtgctcagcctgcaagtctccccacaacctcacagcgaaagaactctgttaa

SEQ ID NO: 57 - DNA, 120 bp, Artificial Sequence; identical to SEQ ID NO: 56
  artificial sequence

SEQ ID NO: 58 - DNA, 120 bp, Artificial Sequence
  artificial sequence
cctttgctccaacagacaggctgggacacgtcagaaagtgagctgagtgagggtgagctggagaggcggcggcggacactcctacagcagctggatgatcaccagtgacccaatgagctg

SEQ ID NO: 59 - DNA, 120 bp, Artificial Sequence; identical to SEQ ID NO: 58
  artificial sequence

SEQ ID NO: 60 - DNA, 120 bp, Artificial Sequence
  artificial sequence
ataatgacccttgtttccctctaggcagagtttacagccatgcgggaccagtatatgagggcaggagaagggtttatcatctgttactctatcacggatcgtcgaagtttccatgaagtt

SEQ ID NO: 61 - DNA, 120 bp, Artificial Sequence
  artificial sequence
taagactgctgtccctccgttgagtgaaggagatgggtattctagtgagaatacatcgcgtgctcatacaccactcaacacacctgatccttccaccaagctgagcacagaagctgacac

SEQ ID NO: 62 - DNA, 120 bp, Artificial Sequence
  artificial sequence
caaagattcagacatatactgtactttgaacgatagcaacccttctttgtgtaactctgaagctgaaaatattgagccttcagttatgaagatttcttcaaatagctttatgaatgtgca

SEQ ID NO: 63 - DNA, 120 bp, Artificial Sequence
  artificial sequence
tcgttcgctttcacgacaagcgcgacgctgaggacgctatggatgccatggacggggccgtgctggacggccgcgagctgcgggtgcaaatggcgcgctacggccgccccccggactcac

SEQ ID NO: 64 - DNA, 120 bp, Artificial Sequence
  artificial sequence
cagcaaacttatcatttatgacattgttgacatgcatgcagctgcagacatcttcaaacactacatgaaggtatagttaaatattcttatttttctccttcctctaactggcagagaaat

SEQ ID NO: 65 - DNA, 120 bp, Artificial Sequence
  artificial sequence
tttttctttctttttcccagcaaattgaagagttttctgatgttaatgaaggagagaaagaagtgatgaaactctggaatctccatgtcatgaagcatgggtagggtatttctaaattaa